European Patent Specification EP 3 745 404 B1, published April 3, 2024. Title: Method and System for predicting coupling probabilities of G-protein coupled receptors. Applicant: Inoue Asuka, Universität Heidelberg. The sequence listing filed with the application follows.

SEQUENCE LISTING (96 sequences)

SEQ ID NO: 1 - protein, 502 aa, Homo sapiens
  DREADD M3D
MDYKDDDDKGSTLHNNSTTSPLFPNISSSWIHSPSDAGLPPGTVTHFGSYNVSRAAGNFSSPDGTTDDPLGGHTVWQVVFIAFLTGILALVTIIGNILVIVSFKVNKQLKTVNNYFLLSLACADLIIGVISMNLFTTYIIMNRWALGNLACDLWLAIDCVASNASVMNLLVISFDRYFSITRPLTYRAKRTTKRAGVMIGLAWVISFVLWAPAILFWQYFVGKRTVPPGECFIQFLSEPTITFGTAIAGFYMPVTIMTILYWRIYKETEKRTKELAGLQASGTEAETENFVHPTGSSRSCSSYELQQQSMKRSNRRKYGRCHFWFTTKSWKPSSEQMDQDHSSSDSWNNNDAAASLENSASSDEEDIGSETRAIYSIVLKLPGHSTILNSTKLPSSDNLQVPEEELGMVDLERKADKLQAQKSVDDGGSFPKSFSKLPIQLESAVDTAKTSDVNSSVGKSTATLPLSFKEATLAKRFALKTRSQITKRKRMSLVKEKKAAQT

SEQ ID NO: 2 - protein, 388 aa, Homo sapiens
  M3D-GPR183/ICL3
MDYKDDDDKGSTLHNNSTTSPLFPNISSSWIHSPSDAGLPPGTVTHFGSYNVSRAAGNFSSPDGTTDDPLGGHTVWQVVFIAFLTGILALVTIIGNILVIVSFKVNKQLKTVNNYFLLSLACADLIIGVISMNLFTTYIIMNRWALGNLACDLWLAIDCVASNASVMNLLVISFDRYFSITRPLTYRAKRTTKRAGVMIGLAWVISFVLWAPAILFWQYFVGKRTVPPGECFIQFLSEPTITFGTAIAGFYMPVTIMTILYWRIYKETERTAKQNPLTEKSGVEKKAAQTLSAILLAFIITWTPYNIMVLVNTFCDSCIPKTFWNLGYWLCYINSTVNPVCYALCNKTFRTTFKMLLLCQCDKKKRRKQQYQQRQSVIFHKRAPEQAL

SEQ ID NO: 3 - protein, 383 aa, Homo sapiens
  M3D-GPR132/ICL3
MDYKDDDDKGSTLHNNSTTSPLFPNISSSWIHSPSDAGLPPGTVTHFGSYNVSRAAGNFSSPDGTTDDPLGGHTVWQVVFIAFLTGILALVTIIGNILVIVSFKVNKQLKTVNNYFLLSLACADLIIGVISMNLFTTYIIMNRWALGNLACDLWLAIDCVASNASVMNLLVISFDRYFSITRPLTYRAKRTTKRAGVMIGLAWVISFVLWAPAILFWQYFVGKRTVPPGECFIQFLSEPTITFGTAIAGFYMPVTIMTILYWRIYKETEQSMGLSAAQEKKAAQTLSAILLAFIITWTPYNIMVLVNTFCDSCIPKTFWNLGYWLCYINSTVNPVCYALCNKTFRTTFKMLLLCQCDKKKRRKQQYQQRQSVIFHKRAPEQAL

SEQ ID NO: 4 - protein, 388 aa, Homo sapiens
  M3D-GPR183/ICL3 (1.57V)
MDYKDDDDKGSTLHNNSTTSPLFPNISSSWIHSPSDAGLPPGTVTHFGSYNVSRAAGNFSSPDGTTDDPLGGHTVWQVVFIAFLTGILALVTIIGNILVIVSVKVNKQLKTVNNYFLLSLACADLIIGVISMNLFTTYIIMNRWALGNLACDLWLAIDCVASNASVMNLLVISFDRYFSITRPLTYRAKRTTKRAGVMIGLAWVISFVLWAPAILFWQYFVGKRTVPPGECFIQFLSEPTITFGTAIAGFYMPVTIMTILYWRIYKETERTAKQNPLTEKSGVEKKAAQTLSAILLAFIITWTPYNIMVLVNTFCDSCIPKTFWNLGYWLCYINSTVNPVCYALCNKTFRTTFKMLLLCQCDKKKRRKQQYQQRQSVIFHKRAPEQAL

SEQ ID NO: 5 - protein, 582 aa, Homo sapiens
  Gαs-Lg (GNAS-LgBiT)
MGCLGNSKTEDQRNEEKAQREANKKIEKQLQKDKQVYRATHRLLLLGAGESGKSTIVKQMRILHVNGFNGEGGEEDPQAARSNSDGEKATKVQDIKNNLKEAIETIVAAMSNLGGSGGGGSGGSSSGGVFTLEDFVGDWEQTAAYNLDQVLEQGGVSSLLQNLAVSVTPIQRIVRSGENALKIDIHVIIPYEGLSADQMAQIEEVFKVVYPVDDHHFKVILPYGTLVIDGVTPNMLNYFGRPYEGIAVFDGKKITVTGTLWNGNKIIDERLITPDGSMLFRVTINSGGSGGGGSGGSSSGGVPPVELANPENQFRVDYILSVMNVPDFDFPPEFYEHAKALWEDEGVRACYERSNEYQLIDCAQYFLDKIDVIKQADYVPSDQDLLRCRVLTSGIFETKFQVDKVNFHMFDVGGQRDERRKWIQCFNDVTAIIFVVASSSYNMVIREDNQTNRLQEALNLFKSIWNNRWLRTISVILFLNKQDLLAEKVLAGKSKIEDYFPEFARYTTPEDATPEPGEDPRVTRAKYFIRDEFLRISTASGDGRHYCYPHFTCAVDTENIRRVFNDCRDIIQRMHLRQYELL

SEQ ID NO: 6 - protein, 542 aa, Homo sapiens
  Gαi1-Lg (GNAI1-LgBiT)
MGCTLSAEDKAAVERSKMIDRNLREDGEKAAREVKLLLLGAGESGKSTIVKQMKIIHEAGYSEEECKQYKAVVYSNTIQSIIAIIRAMGRLGGSGGGGSGGSSSGGVFTLEDFVGDWEQTAAYNLDQVLEQGGVSSLLQNLAVSVTPIQRIVRSGENALKIDIHVIIPYEGLSADQMAQIEEVFKVVYPVDDHHFKVILPYGTLVIDGVTPNMLNYFGRPYEGIAVFDGKKITVTGTLWNGNKIIDERLITPDGSMLFRVTINSGGSGGGGSGGSSSGGKIDFGDSARADDARQLFVLAGAAEEGFMTAELAGVIKRLWKDSGVQACFNRSREYQLNDSAAYYLNDLDRIAQPNYIPTQQDVLRTRVKTTGIVETHFTFKDLHFKMFDVGGQRSERKKWIHCFEGVTAIIFCVALSDYDLVLAEDEEMNRMHESMKLFDSICNNKWFTDTSIILFLNKKDLFEEKIKKSPLTICYPEYAGSNTYEEAAAYIQCQFEDLNKRKDTKEIYTHFTCATDTKNVQFVFDAVTDVIIKNNLKDCGLF

SEQ ID NO: 7 - protein, 543 aa, Homo sapiens
  Gαi2-Lg (GNAI2-LgBiT)
MGCTVSAEDKAAAERSKMIDKNLREDGEKAAREVKLLLLGAGESGKSTIVKQMKIIHEDGYSEEECRQYRAVVYSNTIQSIMAIVKAMGNLGGSGGGGSGGSSSGGVFTLEDFVGDWEQTAAYNLDQVLEQGGVSSLLQNLAVSVTPIQRIVRSGENALKIDIHVIIPYEGLSADQMAQIEEVFKVVYPVDDHHFKVILPYGTLVIDGVTPNMLNYFGRPYEGIAVFDGKKITVTGTLWNGNKIIDERLITPDGSMLFRVTINSGGSGGGGSGGSSSGGQIDFADPSRADDARQLFALSCTAEEQGVLPDDLSGVIRRLWADHGVQACFGRSREYQLNDSAAYYLNDLERIAQSDYIPTQQDVLRTRVKTTGIVETHFTFKDLHFKMFDVGGQRSERKKWIHCFEGVTAIIFCVALSAYDLVLAEDEEMNRMHESMKLFDSICNNKWFTDTSIILFLNKKDLFEEKITHSPLTICFPEYTGANKYDEAASYIQSKFEDLNKRKDTKEIYTHFTCATDTKNVQFVFDAVTDVIIKNNLKDCGLF

SEQ ID NO: 8 - protein, 542 aa, Homo sapiens
  Gαi3-Lg (GNAI3-LgBiT)
MGCTLSAEDKAAVERSKMIDRNLREDGEKAAKEVKLLLLGAGESGKSTIVKQMKIIHEDGYSEDECKQYKVVVYSNTIQSIIAIIRAMGRLGGSGGGGSGGSSSGGVFTLEDFVGDWEQTAAYNLDQVLEQGGVSSLLQNLAVSVTPIQRIVRSGENALKIDIHVIIPYEGLSADQMAQIEEVFKVVYPVDDHHFKVILPYGTLVIDGVTPNMLNYFGRPYEGIAVFDGKKITVTGTLWNGNKIIDERLITPDGSMLFRVTINSGGSGGGGSGGSSSGGKIDFGEAARADDARQLFVLAGSAEEGVMTPELAGVIKRLWRDGGVQACFSRSREYQLNDSASYYLNDLDRISQSNYIPTQQDVLRTRVKTTGIVETHFTFKDLYFKMFDVGGQRSERKKWIHCFEGVTAIIFCVALSDYDLVLAEDEEMNRMHESMKLFDSICNNKWFTETSIILFLNKKDLFEEKIKRSPLTICYPEYTGSNTYEEAAAYIQCQFEDLNRRKDTKEIYTHFTCATDTKNVQFVFDAVTDVIIKNNLKECGLY

SEQ ID NO: 9 - protein, 542 aa, Homo sapiens
  Gαo-Lg (GNAO1-LgBiT)
MGCTLSAEERAALERSKAIEKNLKEDGISAAKDVKLLLLGAGESGKSTIVKQMKIIHEDGFSGEDVKQYKPVVYSNTIQSLAAIVRAMDTLGGSGGGGSGGSSSGGVFTLEDFVGDWEQTAAYNLDQVLEQGGVSSLLQNLAVSVTPIQRIVRSGENALKIDIHVIIPYEGLSADQMAQIEEVFKVVYPVDDHHFKVILPYGTLVIDGVTPNMLNYFGRPYEGIAVFDGKKITVTGTLWNGNKIIDERLITPDGSMLFRVTINSGGSGGGGSGGSSSGGGIEYGDKERKADAKMVCDVVSRMEDTEPFSAELLSAMMRLWGDSGIQECFNRSREYQLNDSAKYYLDSLDRIGAADYQPTEQDILRTRVKTTGIVETHFTFKNLHFRLFDVGGQRSERKKWIHCFEDVTAIIFCVALSGYDQVLHEDETTNRMHESLMLFDSICNNKFFIDTSIILFLNKKDLFGEKIKKSPLTICFPEYTGPNTYEDAAAYIQAQFESKNRSPNKEIYCHMTCATDTNNIQVVFDAVTDIIIANNLRGCGLY

SEQ ID NO: 10 - protein, 547 aa, Homo sapiens
  Gαq-Lg (GNAQ-LgBiT)
MTLESIMACCLSEEAKEARRINDEIERQLRRDKRDARRELKLLLLGTGESGKSTFIKQMRIIHGSGYSDEDKRGFTKLVYQNIFTAMQAMIRAMDTLGGSGGGGSGGSSSGGVFTLEDFVGDWEQTAAYNLDQVLEQGGVSSLLQNLAVSVTPIQRIVRSGENALKIDIHVIIPYEGLSADQMAQIEEVFKVVYPVDDHHFKVILPYGTLVIDGVTPNMLNYFGRPYEGIAVFDGKKITVTGTLWNGNKIIDERLITPDGSMLFRVTINSGGSGGGGSGGSSSGGKIPYKYEHNKAHAQLVREVDVEKVSAFENPYVDAIKSLWNDPGIQECYDRRREYQLSDSTKYYLNDLDRVADPAYLPTQQDVLRVRVPTTGIIEYPFDLQSVIFRMVDVGGQRSERRKWIHCFENVTSIMFLVALSEYDQVLVESDNENRMEESKALFRTIITYPWFQNSSVILFLNKKDLLEEKIMYSHLVDYFPEYDGPQRDAQAAREFILKMFVDLNPDSDKIIYSHFTCATDTENIRFVFAAVKDTILQLNLKEYNLV

SEQ ID NO: 11 - protein, 547 aa, Homo sapiens
  Gα11-Lg (GNA11-LgBiT)
MTLESMMACCLSDEVKESKRINAEIEKQLRRDKRDARRELKLLLLGTGESGKSTFIKQMRIIHGAGYSEEDKRGFTKLVYQNIFTAMQAMIRAMETLGGSGGGGSGGSSSGGVFTLEDFVGDWEQTAAYNLDQVLEQGGVSSLLQNLAVSVTPIQRIVRSGENALKIDIHVIIPYEGLSADQMAQIEEVFKVVYPVDDHHFKVILPYGTLVIDGVTPNMLNYFGRPYEGIAVFDGKKITVTGTLWNGNKIIDERLITPDGSMLFRVTINSGGSGGGGSGGSSSGGKILYKYEQNKANALLIREVDVEKVTTFEHQYVSAIKTLWEDPGIQECYDRRREYQLSDSAKYYLTDVDRIATLGYLPTQQDVLRVRVPTTGIIEYPFDLENIIFRMVDVGGQRSERRKWIHCFENVTSIMFLVALSEYDQVLVESDNENRMEESKALFRTIITYPWFQNSSVILFLNKKDLLEDKILYSHLVDYFPEFDGPQRDAQAAREFILKMFVDLNPDSDKIIYSHFTCATDTENIRFVFAAVKDTILQLNLKEYNLV

SEQ ID NO: 12 - protein, 543 aa, Homo sapiens
  Gα14-Lg (GNA14-LgBiT)
MAGCCCLSAEEKESQRISAEIERQLRRDKKDARRELKLLLLGTGESGKSTFIKQMRIIHGSGYSDEDRKGFTKLVYQNIFTAMQAMIRAMDTLGGSGGGGSGGSSSGGVFTLEDFVGDWEQTAAYNLDQVLEQGGVSSLLQNLAVSVTPIQRIVRSGENALKIDIHVIIPYEGLSADQMAQIEEVFKVVYPVDDHHFKVILPYGTLVIDGVTPNMLNYFGRPYEGIAVFDGKKITVTGTLWNGNKIIDERLITPDGSMLFRVTINSGGSGGGGSGGSSSGGRIQYVCEQNKENAQIIREVEVDKVSMLSREQVEAIKQLWQDPGIQECYDRRREYQLSDSAKYYLTDIDRIATPSFVPTQQDVLRVRVPTTGIIEYPFDLENIIFRMVDVGGQRSERRKWIHCFESVTSIIFLVALSEYDQVLAECDNENRMEESKALFKTIITYPWFLNSSVILFLNKKDLLEEKIMYSHLISYFPEYTGPKQDVRAARDFILKLYQDQNPDKEKVIYSHFTCATDTDNIRFVFAAVKDTILQLNLREFNLV

SEQ ID NO: 13 - protein, 562 aa, Homo sapiens
  Gα16-Lg (GNA15-LgBiT)
MARSLTWRCCPWCLTEDEKAAARVDQEINRILLEQKKQDRGELKLLLLGPGESGKSTFIKQMRIIHGAGYSEEERKGFRPLVYQNIFVSMRAMIEAMERLGGSGGGGSGGSSSGGVFTLEDFVGDWEQTAAYNLDQVLEQGGVSSLLQNLAVSVTPIQRIVRSGENALKIDIHVIIPYEGLSADQMAQIEEVFKVVYPVDDHHFKVILPYGTLVIDGVTPNMLNYFGRPYEGIAVFDGKKITVTGTLWNGNKIIDERLITPDGSMLFRVTINSGGSGGGGSGGSSSGGQIPFSRPESKHHASLVMSQDPYKVTTFEKRYAAAMQWLWRDAGIRAYYERRREFHLLDSAVYYLSHLERITEEGYVPTAQDVLRSRMPTTGINEYCFSVQKTNLRIVDVGGQKSERKKWIHCFENVIALIYLASLSEYDQCLEENNQENRMKESLALFGTILELPWFKSTSVILFLNKTDILEEKIPTSHLATYFPSFQGPKQDAEAAKRFILDMYTRMYTGCVDGPEGSKKGARSRRLFSHYTCATDTQNIRKVFKDVRDSVLARYLDEINLL

SEQ ID NO: 14 - protein, 569 aa, Homo sapiens
  Gα12-Lg (GNA12-LgBiT)
MSGVVRTLSRCLLPAEAGGARERRAGSGARDAEREARRRSRDIDALLARERRAVRRLVKILLLGAGESGKSTFLKQMRIIHGREFDQKALLEFRDTIFDNILKGSRVLVDARDKLGGSGGGGSGGSSSGGVFTLEDFVGDWEQTAAYNLDQVLEQGGVSSLLQNLAVSVTPIQRIVRSGENALKIDIHVIIPYEGLSADQMAQIEEVFKVVYPVDDHHFKVILPYGTLVIDGVTPNMLNYFGRPYEGIAVFDGKKITVTGTLWNGNKIIDERLITPDGSMLFRVTINSGGSGGGGSGGSSSGGGIPWQYSENEKHGMFLMAFENKAGLPVEPATFQLYVPALSALWRDSGIREAFSRRSEFQLGESVKYFLDNLDRIGQLNYFPSKQDILLARKATKGIVEHDFVIKKIPFKMVDVGGQRSQRQKWFQCFDGITSILFMVSSSEYDQVLMEDRRTNRLVESMNIFETIVNNKLFFNVSIILFLNKMDLLVEKVKTVSIKKHFPDFRGDPHRLEDVQRYLVQCFDRKRRNRSKPLFHHFTTAIDTENVRFVFHAVKDTILQENLKDIMLQ

SEQ ID NO: 15 - protein, 565 aa, Homo sapiens
  Gα13-Lg (GNA13-LgBiT)
MADFLPSRSVLSVCFPGCLLTSGEAEQQRKSKEIDKCLSREKTYVKRLVKILLLGAGESGKSTFLKQMRIIHGQDFDQRAREEFRPTIYSNVIKGMRVLVDAREKLGGSGGGGSGGSSSGGVFTLEDFVGDWEQTAAYNLDQVLEQGGVSSLLQNLAVSVTPIQRIVRSGENALKIDIHVIIPYEGLSADQMAQIEEVFKVVYPVDDHHFKVILPYGTLVIDGVTPNMLNYFGRPYEGIAVFDGKKITVTGTLWNGNKIIDERLITPDGSMLFRVTINSGGSGGGGSGGSSSGGHIPWGDNSNQQHGDKMMSFDTRAPMAAQGMVETRVFLQYLPAIRALWADSGIQNAYDRRREFQLGESVKYFLDNLDKLGEPDYIPSQQDILLARRPTKGIHEYDFEIKNVPFKMVDVGGQRSERKRWFECFDSVTSILFLVSSSEFDQVLMEDRLTNRLTESLNIFETIVNNRVFSNVSIILFLNKTDLLEEKVQIVSIKDYFLEFEGDPHCLRDVQKFLVECFRNKRRDQQQKPLYHHFTTAINTENIRLVFRDVKDTILHDNLKQLMLQ

SEQ ID NO: 16 - protein, 366 aa, Homo sapiens
  Sm-Gβ1 (SmBiT-GNB1)
MVTGYRLFEEILGGSGGGGSGGSSSGGSELDQLRQEAEQLKNQIRDARKACADATLSQITNNIDPVGRIQMRTRRTLRGHLAKIYAMHWGTDSRLLVSASQDGKLIIWDSYTTNKVHAIPLRSSWVMTCAYAPSGNYVACGGLDNICSIYNLKTREGNVRVSRELAGHTGYLSCCRFLDDNQIVTSSGDTTCALWDIETGQQTTTFTGHTGDVMSLSLAPDTRLFVSGACDASAKLWDVREGMCRQTFTGHESDINAICFFPNGNAFATGSDDATCRLFDLRADQELMTYSHDNIICGITSVSFSKSGRLLLAGYDDFNCNVWDALKADRAGVLAGHDNRVSCLGVTDDGMAVATGSWDSFLKIWN

SEQ ID NO: 17 - protein, 366 aa, Homo sapiens
  Sm-Gβ2 (SmBiT-GNB2)
MVTGYRLFEEILGGSGGGGSGGSSSGGSELEQLRQEAEQLRNQIRDARKACGDSTLTQITAGLDPVGRIQMRTRRTLRGHLAKIYAMHWGTDSRLLVSASQDGKLIIWDSYTTNKVHAIPLRSSWVMTCAYAPSGNFVACGGLDNICSIYSLKTREGNVRVSRELPGHTGYLSCCRFLDDNQIITSSGDTTCALWDIETGQQTVGFAGHSGDVMSLSLAPDGRTFVSGACDASIKLWDVRDSMCRQTFIGHESDINAVAFFPNGYAFTTGSDDATCRLFDLRADQELLMYSHDNIICGITSVAFSRSGRLLLAGYDDFNCNIWDAMKGDRAGVLAGHDNRVSCLGVTDDGMAVATGSWDSFLKIWN

SEQ ID NO: 18 - protein, 366 aa, Homo sapiens
  Sm-Gβ3 (SmBiT-GNB3)
MVTGYRLFEEILGGSGGGGSGGSSSGGGEMEQLRQEAEQLKKQIADARKACADVTLAELVSGLEVVGRVQMRTRRTLRGHLAKIYAMHWATDSKLLVSASQDGKLIVWDSYTTNKVHAIPLRSSWVMTCAYAPSGNFVACGGLDNMCSIYNLKSREGNVKVSRELSAHTGYLSCCRFLDDNNIVTSSGDTTCALWDIETGQQKTVFVGHTGDCMSLAVSPDFNLFISGACDASAKLWDVREGTCRQTFTGHESDINAICFFPNGEAICTGSDDASCRLFDLRADQELICFSHESIICGITSVAFSLSGRLLFAGYDDFNCNVWDSMKSERVGILSGHDNRVSCLGVTADGMAVATGSWDSFLKIWN

SEQ ID NO: 19 - protein, 366 aa, Homo sapiens
  Sm-Gβ4 (SmBiT-GNB4)
MVTGYRLFEEILGGSGGGGSGGSSSGGSELEQLRQEAEQLRNQIQDARKACNDATLVQITSNMDSVGRIQMRTRRTLRGHLAKIYAMHWGYDSRLLVSASQDGKLIIWDSYTTNKMHAIPLRSSWVMTCAYAPSGNYVACGGLDNICSIYNLKTREGNVRVSRELPGHTGYLSCCRFLDDSQIVTSSGDTTCALWDIETAQQTTTFTGHSGDVMSLSLSPDMRTFVSGACDASSKLWDIRDGMCRQSFTGHVSDINAVSFFPNGYAFATGSDDATCRLFDLRADQELLLYSHDNIICGITSVAFSKSGRLLLAGYDDFNCNVWDTLKGDRAGVLAGHDNRVSCLGVTDDGMAVATGSWDSFLRIWN

SEQ ID NO: 20 - protein, 421 aa, Homo sapiens
  Sm-Gβ5 (SmBiT-GNB5)
MVTGYRLFEEILGGSGGGGSGGSSSGGCDQTFLVNVFGSCDKCFKQRALRPVFKKSQQLSYCSTCAEIMATEGLHENETLASLKSEAESLKGKLEEERAKLHDVELHQVAERVEALGQFVMKTRRTLKGHGNKVLCMDWCKDKRRIVSSSQDGKVIVWDSFTTNKEHAVTMPCTWVMACAYAPSGCAIACGGLDNKCSVYPLTFDKNENMAAKKKSVAMHTNYLSACSFTNSDMQILTASGDGTCALWDVESGQLLQSFHGHGADVLCLDLAPSETGNTFVSGGCDKKAMVWDMRSGQCVQAFETHESDINSVRYYPSGDAFASGSDDATCRLYDLRADREVAIYSKESIIFGASSVDFSLSGRLLFAGYNDYTINVWDVLKGSRVSILFGHENRVSTLRVSPDGTAFCSGSWDHTLRVWA

SEQ ID NO: 21 - protein, 97 aa, Homo sapiens
  Sm-Gγ2 (SmBiT-GNG2)
MVTGYRLFEEILGGSGGGGSGGSSSGGASNNTASIAQARKLVEQLKMEANIDRIKVSKAAADLMAYCEAHAKEDPLLTPVPASENPFREKKFFCAIL

SEQ ID NO: 22 - protein, 101 aa, Homo sapiens
  Sm-Gγ3 (SmBiT-GNG3)
MVTGYRLFEEILGGSGGGGSGGSSSGGKGETPVNSTMSIGQARKMVEQLKIEASLCRIKVSKAAADLMTYCDAHACEDPLITPVPTSENPFREKKFFCALL

SEQ ID NO: 23 - protein, 101 aa, Homo sapiens
  Sm-Gγ4 (SmBiT-GNG4)
MVTGYRLFEEILGGSGGGGSGGSSSGGKEGMSNNSTTSISQARKAVEQLKMEACMDRVKVSQAAADLLAYCEAHVREDPLIIPVPASENPFREKKFFCTIL

SEQ ID NO: 24 - protein, 94 aa, Homo sapiens
  Sm-Gγ5 (SmBiT-GNG5)
MVTGYRLFEEILGGSGGGGSGGSSSGGSGSSSVAAMKKVVQQLRLEAGLNRVKVSQAAADLKQFCLQNAQHDPLLTGVSSSTNPFRPQKVCSFL

SEQ ID NO: 25 - protein, 94 aa, Homo sapiens
  Sm-Gγ7 (SmBiT-GNG7)
MVTGYRLFEEILGGSGGGGSGGSSSGGSATNNIAQARKLVEQLRIEAGIERIKVSKAASDLMSYCEQHARNDPLLVGVPASENPFKDKKPCIIL

SEQ ID NO: 26 - protein, 96 aa, Homo sapiens
  Sm-Gγ8 (SmBiT-GNG8)
MVTGYRLFEEILGGSGGGGSGGSSSGGSNNMAKIAEARKTVEQLKLEVNIDRMKVSQAAAELLAFCETHAKDDPLVTPVPAAENPFRDKRLFCVLL

SEQ ID NO: 27 - protein, 94 aa, Homo sapiens
  Sm-Gγ10 (SmBiT-GNG10)
MVTGYRLFEEILGGSGGGGSGGSSSGGSSGASASALQRLVEQLKLEAGVERIKVSQAAAELQQYCMQNACKDALLVGVPAGSNPFREPRSCALL

SEQ ID NO: 28 - protein, 99 aa, Homo sapiens
  Sm-Gγ11 (SmBiT-GNG11)
MVTGYRLFEEILGGSGGGGSGGSSSGGPALHIEDLPEKEKLKMEVEQLRKEVKLQRQQVSKCSEEIKNYIEERSGEDPLVKGIPEDKNPFKEKGSCVIS

SEQ ID NO: 29 - protein, 98 aa, Homo sapiens
  Sm-Gγ12 (SmBiT-GNG12)
MVTGYRLFEEILGGSGGGGSGGSSSGGSSKTASTNNIAQARRTVQQLRLEASIERIKVSKASADLMSYCEEHARSDPLLIGIPTSENPFKDKKTCIIL

SEQ ID NO: 30 - protein, 93 aa, Homo sapiens
  Sm-Gγ13 (SmBiT-GNG13)
MVTGYRLFEEILGGSGGGGSGGSSSGGEEWDVPQMKKEVESLKYQLAFQREMASKTIPELLKWIEDGIPKDPFLNPDLMKNNPWVEKGKCTIL

SEQ ID NO: 31 - protein, 100 aa, Homo sapiens
  Sm-Gγt1 (SmBiT-GNGT1)
MVTGYRLFEEILGGSGGGGSGGSSSGGPVINIEDLTEKDKLKMEVDQLKKEVTLERMLVSKCCEEVRDYVEERSGEDPLVKGIPEDKNPFKELKGGCVIS

SEQ ID NO: 32 - protein, 95 aa, Homo sapiens
  Sm-Gγ (SmBiT-GNGT2)
MVTGYRLFEEILGGSGGGGSGGSSSGGAQDLSEKDLLKMEVEQLKKEVKNTRIPISKAGKEIKEYVEAQAGNDPFLKGIPEDKNPFKEKGGCLIS

SEQ ID NO: 33 - protein, 435 aa, Homo sapiens
  Gαs-Sm (GNAS-SmBiT)
MGCLGNSKTEDQRNEEKAQREANKKIEKQLQKDKQVYRATHRLLLLGAGESGKSTIVKQMRILHVNGFNGEGGEEDPQAARSNSDGEKATKVQDIKNNLKEAIETIVAAMSNLGGSGGGGSGGSSSGGVTGYRLFEEILGGSGGGGSGGSSSGGVPPVELANPENQFRVDYILSVMNVPDFDFPPEFYEHAKALWEDEGVRACYERSNEYQLIDCAQYFLDKIDVIKQADYVPSDQDLLRCRVLTSGIFETKFQVDKVNFHMFDVGGQRDERRKWIQCFNDVTAIIFVVASSSYNMVIREDNQTNRLQEALNLFKSIWNNRWLRTISVILFLNKQDLLAEKVLAGKSKIEDYFPEFARYTTPEDATPEPGEDPRVTRAKYFIRDEFLRISTASGDGRHYCYPHFTCAVDTENIRRVFNDCRDIIQRMHLRQYELL

SEQ ID NO: 34 - protein, 568 aa, Homo sapiens
  Gαs-Lg (αB-αC) (GNAS-LgBiT-αB-αC)
MGCLGNSKTEDQRNEEKAQREANKKIEKQLQKDKQVYRATHRLLLLGAGESGKSTIVKQMRILHVNGFNGDSEKATKVQDIKNNLKEAIETIVAAMSNLVPPVELANPENQFRVDYILSVMNVPDFGGSGGGGSGGSSSGGVFTLEDFVGDWEQTAAYNLDQVLEQGGVSSLLQNLAVSVTPIQRIVRSGENALKIDIHVIIPYEGLSADQMAQIEEVFKVVYPVDDHHFKVILPYGTLVIDGVTPNMLNYFGRPYEGIAVFDGKKITVTGTLWNGNKIIDERLITPDGSMLFRVTINSGGSGGGGSGGSSSGGDFPPEFYEHAKALWEDEGVRACYERSNEYQLIDCAQYFLDKIDVIKQADYVPSDQDLLRCRVLTSGIFETKFQVDKVNFHMFDVGGQRDERRKWIQCFNDVTAIIFVVASSSYNMVIREDNQTNRLQEALNLFKSIWNNRWLRTISVILFLNKQDLLAEKVLAGKSKIEDYFPEFARYTTPEDATPEPGEDPRVTRAKYFIRDEFLRISTASGDGRHYCYPHFTCAVDTENIRRVFNDCRDIIQRMHLRQYELL

SEQ ID NO: 35 - protein, 421 aa, Homo sapiens
  Gαs-Sm (αB-αC) (GNAS-SmBiT-αB-αC)
MGCLGNSKTEDQRNEEKAQREANKKIEKQLQKDKQVYRATHRLLLLGAGESGKSTIVKQMRILHVNGFNGDSEKATKVQDIKNNLKEAIETIVAAMSNLVPPVELANPENQFRVDYILSVMNVPDFGGSGGGGSGGSSSGGVTGYRLFEEILGGSGGGGSGGSSSGGDFPPEFYEHAKALWEDEGVRACYERSNEYQLIDCAQYFLDKIDVIKQADYVPSDQDLLRCRVLTSGIFETKFQVDKVNFHMFDVGGQRDERRKWIQCFNDVTAIIFVVASSSYNMVIREDNQTNRLQEALNLFKSIWNNRWLRTISVILFLNKQDLLAEKVLAGKSKIEDYFPEFARYTTPEDATPEPGEDPRVTRAKYFIRDEFLRISTASGDGRHYCYPHFTCAVDTENIRRVFNDCRDIIQRMHLRQYELL

SEQ ID NO: 36 - protein, 582 aa, Homo sapiens
  Gαs-Lg (G2A/C3S) (GNAS-LgBiT-G2A-C3S)
MASLGNSKTEDQRNEEKAQREANKKIEKQLQKDKQVYRATHRLLLLGAGESGKSTIVKQMRILHVNGFNGEGGEEDPQAARSNSDGEKATKVQDIKNNLKEAIETIVAAMSNLGGSGGGGSGGSSSGGVFTLEDFVGDWEQTAAYNLDQVLEQGGVSSLLQNLAVSVTPIQRIVRSGENALKIDIHVIIPYEGLSADQMAQIEEVFKVVYPVDDHHFKVILPYGTLVIDGVTPNMLNYFGRPYEGIAVFDGKKITVTGTLWNGNKIIDERLITPDGSMLFRVTINSGGSGGGGSGGSSSGGVPPVELANPENQFRVDYILSVMNVPDFDFPPEFYEHAKALWEDEGVRACYERSNEYQLIDCAQYFLDKIDVIKQADYVPSDQDLLRCRVLTSGIFETKFQVDKVNFHMFDVGGQRDERRKWIQCFNDVTAIIFVVASSSYNMVIREDNQTNRLQEALNLFKSIWNNRWLRTISVILFLNKQDLLAEKVLAGKSKIEDYFPEFARYTTPEDATPEPGEDPRVTRAKYFIRDEFLRISTASGDGRHYCYPHFTCAVDTENIRRVFNDCRDIIQRMHLRQYELL

SEQ ID NO: 37 - protein, 547 aa, Homo sapiens
  Gαq-Lg (R183C) (GNAQ-LgBiT-R183C)
MTLESIMACCLSEEAKEARRINDEIERQLRRDKRDARRELKLLLLGTGESGKSTFIKQMRIIHGSGYSDEDKRGFTKLVYQNIFTAMQAMIRAMDTLGGSGGGGSGGSSSGGVFTLEDFVGDWEQTAAYNLDQVLEQGGVSSLLQNLAVSVTPIQRIVRSGENALKIDIHVIIPYEGLSADQMAQIEEVFKVVYPVDDHHFKVILPYGTLVIDGVTPNMLNYFGRPYEGIAVFDGKKITVTGTLWNGNKIIDERLITPDGSMLFRVTINSGGSGGGGSGGSSSGGKIPYKYEHNKAHAQLVREVDVEKVSAFENPYVDAIKSLWNDPGIQECYDRRREYQLSDSTKYYLNDLDRVADPAYLPTQQDVLRVCVPTTGIIEYPFDLQSVIFRMVDVGGQRSERRKWIHCFENVTSIMFLVALSEYDQVLVESDNENRMEESKALFRTIITYPWFQNSSVILFLNKKDLLEEKIMYSHLVDYFPEYDGPQRDAQAAREFILKMFVDLNPDSDKIIYSHFTCATDTENIRFVFAAVKDTILQLNLKEYNLV

SEQ ID NO: 38 - protein, 547 aa, Homo sapiens
  Gαq-Lg (αB-αC) (GNAQ-LgBiT-αB-αC)
MTLESIMACCLSEEAKEARRINDEIERQLRRDKRDARRELKLLLLGTGESGKSTFIKQMRIIHGSGYSDEDKRGFTKLVYQNIFTAMQAMIRAMDTLKIPYKYEHNKAHAQLVREVDVEKVSAGGSGGGGSGGSSSGGVFTLEDFVGDWEQTAAYNLDQVLEQGGVSSLLQNLAVSVTPIQRIVRSGENALKIDIHVIIPYEGLSADQMAQIEEVFKVVYPVDDHHFKVILPYGTLVIDGVTPNMLNYFGRPYEGIAVFDGKKITVTGTLWNGNKIIDERLITPDGSMLFRVTINSGGSGGGGSGGSSSGGFENPYVDAIKSLWNDPGIQECYDRRREYQLSDSTKYYLNDLDRVADPAYLPTQQDVLRVRVPTTGIIEYPFDLQSVIFRMVDVGGQRSERRKWIHCFENVTSIMFLVALSEYDQVLVESDNENRMEESKALFRTIITYPWFQNSSVILFLNKKDLLEEKIMYSHLVDYFPEYDGPQRDAQAAREFILKMFVDLNPDSDKIIYSHFTCATDTENIRFVFAAVKDTILQLNLKEYNLV

SEQ ID NO: 39 - protein, 547 aa, Homo sapiens
  Gα11-Lg (αB-αC) (GNA11-LgBiT-αB-αC)
MTLESMMACCLSDEVKESKRINAEIEKQLRRDKRDARRELKLLLLGTGESGKSTFIKQMRIIHGAGYSEEDKRGFTKLVYQNIFTAMQAMIRAMETLKILYKYEQNKANALLIREVDVEKVTTGGSGGGGSGGSSSGGVFTLEDFVGDWEQTAAYNLDQVLEQGGVSSLLQNLAVSVTPIQRIVRSGENALKIDIHVIIPYEGLSADQMAQIEEVFKVVYPVDDHHFKVILPYGTLVIDGVTPNMLNYFGRPYEGIAVFDGKKITVTGTLWNGNKIIDERLITPDGSMLFRVTINSGGSGGGGSGGSSSGGFEHQYVSAIKTLWEDPGIQECYDRRREYQLSDSAKYYLTDVDRIATLGYLPTQQDVLRVRVPTTGIIEYPFDLENIIFRMVDVGGQRSERRKWIHCFENVTSIMFLVALSEYDQVLVESDNENRMEESKALFRTIITYPWFQNSSVILFLNKKDLLEDKILYSHLVDYFPEFDGPQRDAQAAREFILKMFVDLNPDSDKIIYSHFTCATDTENIRFVFAAVKDTILQLNLKEYNLV

SEQ ID NO: 40 - protein, 543 aa, Homo sapiens
  Gα14-Lg (αB-αC) (GNA14-LgBiT-αB-αC)
MAGCCCLSAEEKESQRISAEIERQLRRDKKDARRELKLLLLGTGESGKSTFIKQMRIIHGSGYSDEDRKGFTKLVYQNIFTAMQAMIRAMDTLRIQYVCEQNKENAQIIREVEVDKVSMGGSGGGGSGGSSSGGVFTLEDFVGDWEQTAAYNLDQVLEQGGVSSLLQNLAVSVTPIQRIVRSGENALKIDIHVIIPYEGLSADQMAQIEEVFKVVYPVDDHHFKVILPYGTLVIDGVTPNMLNYFGRPYEGIAVFDGKKITVTGTLWNGNKIIDERLITPDGSMLFRVTINSGGSGGGGSGGSSSGGLSREQVEAIKQLWQDPGIQECYDRRREYQLSDSAKYYLTDIDRIATPSFVPTQQDVLRVRVPTTGIIEYPFDLENIIFRMVDVGGQRSERRKWIHCFESVTSIIFLVALSEYDQVLAECDNENRMEESKALFKTIITYPWFLNSSVILFLNKKDLLEEKIMYSHLISYFPEYTGPKQDVRAARDFILKLYQDQNPDKEKVIYSHFTCATDTDNIRFVFAAVKDTILQLNLREFNLV

SEQ ID NO: 41 - protein, 562 aa, Homo sapiens
  Gα16-Lg (αB-αC) (GNA15-LgBiT-αB-αC)
MARSLTWRCCPWCLTEDEKAAARVDQEINRILLEQKKQDRGELKLLLLGPGESGKSTFIKQMRIIHGAGYSEEERKGFRPLVYQNIFVSMRAMIEAMERLQIPFSRPESKHHASLVMSQDPYKVTTGGSGGGGSGGSSSGGVFTLEDFVGDWEQTAAYNLDQVLEQGGVSSLLQNLAVSVTPIQRIVRSGENALKIDIHVIIPYEGLSADQMAQIEEVFKVVYPVDDHHFKVILPYGTLVIDGVTPNMLNYFGRPYEGIAVFDGKKITVTGTLWNGNKIIDERLITPDGSMLFRVTINSGGSGGGGSGGSSSGGFEKRYAAAMQWLWRDAGIRAYYERRREFHLLDSAVYYLSHLERITEEGYVPTAQDVLRSRMPTTGINEYCFSVQKTNLRIVDVGGQKSERKKWIHCFENVIALIYLASLSEYDQCLEENNQENRMKESLALFGTILELPWFKSTSVILFLNKTDILEEKIPTSHLATYFPSFQGPKQDAEAAKRFILDMYTRMYTGCVDGPEGSKKGARSRRLFSHYTCATDTQNIRKVFKDVRDSVLARYLDEINLL

SEQ ID NO: 42 - protein, 513 aa, Homo sapiens
  Lg-Gβ1 (LgBiT-GNB1)
MVFTLEDFVGDWEQTAAYNLDQVLEQGGVSSLLQNLAVSVTPIQRIVRSGENALKIDIHVIIPYEGLSADQMAQIEEVFKVVYPVDDHHFKVILPYGTLVIDGVTPNMLNYFGRPYEGIAVFDGKKITVTGTLWNGNKIIDERLITPDGSMLFRVTINSGGSGGGGSGGSSSGGSELDQLRQEAEQLKNQIRDARKACADATLSQITNNIDPVGRIQMRTRRTLRGHLAKIYAMHWGTDSRLLVSASQDGKLIIWDSYTTNKVHAIPLRSSWVMTCAYAPSGNYVACGGLDNICSIYNLKTREGNVRVSRELAGHTGYLSCCRFLDDNQIVTSSGDTTCALWDIETGQQTTTFTGHTGDVMSLSLAPDTRLFVSGACDASAKLWDVREGMCRQTFTGHESDINAICFFPNGNAFATGSDDATCRLFDLRADQELMTYSHDNIICGITSVSFSKSGRLLLAGYDDFNCNVWDALKADRAGVLAGHDNRVSCLGVTDDGMAVATGSWDSFLKIWN

SEQ ID NO: 43 - protein, 244 aa, Homo sapiens
  Lg-Gγ2 (LgBiT-GNG2)
MVFTLEDFVGDWEQTAAYNLDQVLEQGGVSSLLQNLAVSVTPIQRIVRSGENALKIDIHVIIPYEGLSADQMAQIEEVFKVVYPVDDHHFKVILPYGTLVIDGVTPNMLNYFGRPYEGIAVFDGKKITVTGTLWNGNKIIDERLITPDGSMLFRVTINSGGSGGGGSGGSSSGGASNNTASIAQARKLVEQLKMEANIDRIKVSKAAADLMAYCEAHAKEDPLLTPVPASENPFREKKFFCAIL

SEQ ID NO: 44 - protein, 97 aa, Homo sapiens
  Sm-Gγ2 (C68S) (SmBiT-GNG2-C68S)
MVTGYRLFEEILGGSGGGGSGGSSSGGASNNTASIAQARKLVEQLKMEANIDRIKVSKAAADLMAYCEAHAKEDPLLTPVPASENPFREKKFFSAIL

SEQ ID NO: 45 - protein, 1242 aa, Homo sapiens
  Sm-PLCβ1 (SmBiT-PLCB1)
MVTGYRLFEEILGGSGGGGSGGSSSGGAGAQPGVHALQLKPVCVSDSLKKGTKFVKWDDDSTIVTPIILRTDPQGFFFYWTDQNKETELLDLSLVKDARCGRHAKAPKDPKLRELLDVGNIGRLEQRMITVVYGPDLVNISHLNLVAFQEEVAKEWTNEVFSLATNLLAQNMSRDAFLEKAYTKLKLQVTPEGRIPLKNIYRLFSADRKRVETALEACSLPSSRNDSIPQEDFTPEVYRVFLNNLCPRPEIDNIFSEFGAKSKPYLTVDQMMDFINLKQRDPRLNEILYPPLKQEQVQVLIEKYEPNNSLARKGQISVDGFMRYLSGEENGVVSPEKLDLNEDMSQPLSHYFINSSHNTYLTAGQLAGNSSVEMYRQVLLSGCRCVELDCWKGRTAEEEPVITHGFTMTTEISFKEVIEAIAECAFKTSPFPILLSFENHVDSPKQQAKMAEYCRLIFGDALLMEPLEKYPLESGVPLPSPMDLMYKILVKNKKKSHKSSEGSGKKKLSEQASNTYSDSSSMFEPSSPGAGEADTESDDDDDDDDCKKSSMDEGTAGSEAMATEEMSNLVNYIQPVKFESFEISKKRNKSFEMSSFVETKGLEQLTKSPVEFVEYNKMQLSRIYPKGTRVDSSNYMPQLFWNAGCQMVALNFQTMDLAMQINMGMYEYNGKSGYRLKPEFMRRPDKHFDPFTEGIVDGIVANTLSVKIISGQFLSDKKVGTYVEVDMFGLPVDTRRKAFKTKTSQGNAVNPVWEEEPIVFKKVVLPTLACLRIAVYEEGGKFIGHRILPVQAIRPGYHYICLRNERNQPLTLPAVFVYIEVKDYVPDTYADVIEALSNPIRYVNLMEQRAKQLAALTLEDEEEVKKEADPGETPSEAPSEARTTPAENGVNHTTTLTPKPPSQALHSQPAPGSVKAPAKTEDLIQSVLTEVEAQTIEELKQQKSFVKLQKKHYKEMKDLVKRHHKKTTDLIKEHTTKYNEIQNDYLRRRAALEKSAKKDSKKKSEPSSPDHGSSTIEQDLAALDAEMTQKLIDLKDKQQQQLLNLRQEQYYSEKYQKREHIKLLIQKLTDVAEECQNNQLKKLKEICEKEKKELKKKMDKKRQEKITEAKSKDKSQMEEEKTEMIRSYIQEVVQYIKRLEEAQSKRQEKLVEKHKEIRQQILDEKPKLQVELEQEYQDKFKRLPLEILEFVQEAMKGKISEDSNHGSAPLSLSSDPGKVNHKTPSSEELGGDIPGKEFDTPL

SEQ ID NO: 46 - protein, 1207 aa, Homo sapiens
  Sm-PLCβ2 (SmBiT-PLCB2)
MVTGYRLFEEILGGSGGGGSGGSSSGGSLLNPVLLPPKVKAYLSQGERFIKWDDETTVASPVILRVDPKGYYLYWTYQSKEMEFLDITSIRDTRFGKFAKMPKSQKLRDVFNMDFPDNSFLLKTLTVVSGPDMVDLTFHNFVSYKENVGKAWAEDVLALVKHPLTANASRSTFLDKILVKLKMQLNSEGKIPVKNFFQMFPADRKRVEAALSACHLPKGKNDAINPEDFPEPVYKSFLMSLCPRPEIDEIFTSYHAKAKPYMTKEHLTKFINQKQRDSRLNSLLFPPARPDQVQGLIDKYEPSGINAQRGQLSPEGMVWFLCGPENSVLAQDKLLLHHDMTQPLNHYFINSSHNTYLTAGQFSGLSSAEMYRQVLLSGCRCVELDCWKGKPPDEEPIITHGFTMTTDIFFKEAIEAIAESAFKTSPYPIILSFENHVDSPRQQAKMAEYCRTIFGDMLLTEPLEKFPLKPGVPLPSPEDLRGKILIKNKKNQFSGPTSSSKDTGGEAEGSSPPSAPAVWAGEEGTELEEEEVEEEEEEESGNLDEEEIKKMQSDEGTAGLEVTAYEEMSSLVNYIQPTKFVSFEFSAQKNRSYVISSFTELKAYDLLSKASVQFVDYNKRQMSRIYPKGTRMDSSNYMPQMFWNAGCQMVALNFQTMDLPMQQNMAVFEFNGQSGYLLKHEFMRRPDKQFNPFSVDRIDVVVATTLSITVISGQFLSERSVRTYVEVELFGLPGDPKRRYRTKLSPSTNSINPVWKEEPFVFEKILMPELASLRVAVMEEGNKFLGHRIIPINALNSGYHHLCLHSESNMPLTMPALFIFLEMKDYIPGAWADLTVALANPIKFFSAHDTKSVKLKEAMGGLPEKPFPLASPVASQVNGALAPTSNGSPAARAGAREEAMKEAAEPRTASLEELRELKGVVKLQRRHEKELRELERRGARRWEELLQRGAAQLAELGPPGVGGVGACKLGPGKGSRKKRSLPREESAGAAPGEGPEGVDGRVRELKDRLELELLRQGEEQYECVLKRKEQHVAEQISKMMELAREKQAAELKALKETSENDTKEMKKKLETKRLERIQGMTKVTTDKMAQERLKREINNSHIQEVVQVIKQMTENLERHQEKLEEKQAACLEQIREMEKQFQKEALAEYEARMKGLEAEVKESVRACLRTCFPSEAKDKPERACECPPELCEQDPLIAKADAQESRL

SEQ ID NO: 47 - protein, 1260 aa, Homo sapiens
  Sm-PLCβ3 (SmBiT-PLCB3)
MVTGYRLFEEILGGSGGGGSGGSSSGGAGAQPGVHALQLEPPTVVETLRRGSKFIKWDEETSSRNLVTLRVDPNGFFLYWTGPNMEVDTLDISSIRDTRTGRYARLPKDPKIREVLGFGGPDARLEEKLMTVVSGPDPVNTVFLNFMAVQDDTAKVWSEELFKLAMNILAQNASRNTFLRKAYTKLKLQVNQDGRIPVKNILKMFSADKKRVETALESCGLKFNRSESIRPDEFSLEIFERFLNKLCLRPDIDKILLEIGAKGKPYLTLEQLMDFINQKQRDPRLNEVLYPPLRPSQARLLIEKYEPNQQFLERDQMSMEGFSRYLGGEENGILPLEALDLSTDMTQPLSAYFINSSHNTYLTAGQLAGTSSVEMYRQALLWGCRCVELDVWKGRPPEEEPFITHGFTMTTEVPLRDVLEAIAETAFKTSPYPVILSFENHVDSAKQQAKMAEYCRSIFGDALLIEPLDKYPLAPGVPLPSPQDLMGRILVKNKKRHRPSAGGPDSAGRKRPLEQSNSALSESSAATEPSSPQLGSPSSDSCPGLSNGEEVGLEKPSLEPQKSLGDEGLNRGPYVLGPADREDEEEDEEEEEQTDPKKPTTDEGTASSEVNATEEMSTLVNYIEPVKFKSFEAARKRNKCFEMSSFVETKAMEQLTKSPMEFVEYNKQQLSRIYPKGTRVDSSNYMPQLFWNVGCQLVALNFQTLDVAMQLNAGVFEYNGRSGYLLKPEFMRRPDKSFDPFTEVIVDGIVANALRVKVISGQFLSDRKVGIYVEVDMFGLPVDTRRKYRTRTSQGNSFNPVWDEEPFDFPKVVLPTLASLRIAAFEEGGKFVGHRILPVSAIRSGYHYVCLRNEANQPLCLPALLIYTEASDYIPDDHQDYAEALINPIKHVSLMDQRARQLAALIGESEAQAGQETCQDTQSQQLGSQPSSNPTPSPLDASPRRPPGPTTSPASTSLSSPGQRDDLIASILSEVAPTPLDELRGHKALVKLRSRQERDLRELRKKHQRKAVTLTRRLLDGLAQAQAEGRCRLRPGALGGAADVEDTKEGEDEAKRYQEFQNRQVQSLLELREAQVDAEAQRRLEHLRQALQRLREVVLDANTTQFKRLKEMNEREKKELQKILDRKRHNSISEAKMRDKHKKEAELTEINRRHITESVNSIRRLEEAQKQRHDRLVAGQQQVLQQLAEEEPKLLAQLAQECQEQRARLPQEIRRSLLGEMPEGLGDGPLVACASNGHAPGSSGHLSGADSESQEENTQL

SEQ ID NO: 48 - protein, 1220 aa, Homo sapiens
  Sm-PLCβ4 (SmBiT-PLCB4)
MVTGYRLFEEILGGSGGGGSGGSSSGGAKPYEFNWQKEVPSFLQEGAVFDRYEEESFVFEPNCLFKVDEFGFFLTWRSEGKEGQVLECSLINSIRSGAIPKDPKILAALEAVGKSENDLEGRIVCVCSGTDLVNISFTYMVAENPEVTKQWVEGLRSIIHNFRANNVSPMTCLKKHWMKLAFMTNTNGKIPVRSITRTFASGKTEKVIFQALKELGLPSGKNDEIEPTAFSYEKFYELTQKICPRTDIEDLFKKINGDKTDYLTVDQLVSFLNEHQRDPRLNEILFPFYDAKRAMQIIEMYEPDEDLKKKGLISSDGFCRYLMSDENAPVFLDRLELYQEMDHPLAHYFISSSHNTYLTGRQFGGKSSVEMYRQVLLAGCRCVELDCWDGKGEDQEPIITHGKAMCTDILFKDVIQAIKETAFVTSEYPVILSFENHCSKYQQYKMSKYCEDLFGDLLLKQALESHPLEPGRALPSPNDLKRKILIKNKRLKPEVEKKQLEALRSMMEAGESASPANILEDDNEEEIESADQEEEAHPEFKFGNELSADDLGHKEAVANSVKKGLVTVEDEQAWMASYKYVGATTNIHPYLSTMINYAQPVKFQGFHVAEERNIHYNMSSFNESVGLGYLKTHAIEFVNYNKRQMSRIYPKGGRVDSSNYMPQIFWNAGCQMVSLNYQTPDLAMQLNQGKFEYNGSCGYLLKPDFMRRPDRTFDPFSETPVDGVIAATCSVQVISGQFLSDKKIGTYVEVDMYGLPTDTIRKEFRTRMVMNNGLNPVYNEESFVFRKVILPDLAVLRIAVYDDNNKLIGQRILPLDGLQAGYRHISLRNEGNKPLSLPTIFCNIVLKTYVPDGFGDIVDALSDPKKFLSITEKRADQMRAMGIETSDIADVPSDTSKNDKKGKANTAKANVTPQSSSELRPTTTAALASGVEAKKGIELIPQVRIEDLKQMKAYLKHLKKQQKELNSLKKKHAKEHSTMQKLHCTQVDKIVAQYDKEKSTHEKILEKAMKKKGGSNCLEMKKETEIKIQTLTSDHKSKVKEIVAQHTKEWSEMINTHSAEEQEIRDLHLSQQCELLKKLLINAHEQQTQQLKLSHDRESKEMRAHQAKISMENSKAISQDKSIKNKAERERRVRELNSSNTKKFLEERKRLAMKQSKEMDQLKKVQLEHLEFLEKQNEQLLKSCHAVSQTQGEGDAADGEIGSRDGPQTSNSSMKLQNAN

SEQ ID NO: 49 - protein, 158 aa, Homo sapiens
  LgBiT luciferase fragment
VFTLEDFVGDWEQTAAYNLDQVLEQGGVSSLLQNLAVSVTPIQRIVRSGENALKIDIHVIIPYEGLSADQMAQIEEVFKVVYPVDDHHFKVILPYGTLVIDGVTPNMLNYFGRPYEGIAVFDGKKITVTGTLWNGNKIIDERLITPDGSMLFRVTINS

SEQ ID NO: 50 - protein, 12 aa, Homo sapiens
MVTGYRLFEEIL

SEQ ID NO: 51 - protein, 15 aa, Homo sapiens
GGSGGGGSGGSSSGG

SEQ ID NO: 52 - protein, 8 aa, Homo sapiens
DYKDDDDK

SEQ ID NO: 53 - protein, 14 aa, Homo sapiens
  Flag epitope DREADD without linker GS / GSG
RTAKQNPLTEKSGV

SEQ ID NO: 54 - protein, 9 aa, Homo sapiens
QSMGLSAAQ

SEQ ID NO: 55 - protein, 367 aa, Homo sapiens
  Lg-RhoA (LgBiT-RHOA)
MVFTLEDFVGDWEQTAAYNLDQVLEQGGVSSLLQNLAVSVTPIQRIVRSGENALKIDIHVIIPYEGLSADQMAQIEEVFKVVYPVDDHHFKVILPYGTLVIDGVTPNMLNYFGRPYEGIAVFDGKKITVTGTLWNGNKIIDERLITPDGSMLFRVTINSGGSGGGGSGGSSSGGTAAIRKKLVIVGDGACGKTCLLIVFSKDQFPEVYVPTVFENYVADIEVDGKQVELALWDTAGQEDYDRLRPLSYPDTDVILMCFSIDSPDSLENIPEKWTPEVKHFCPNVPIILVGNKKDLRNDEHTRRELAKMKQEPVKPEEGRDMANRIGAFGYMECSAKTKDGVREVFEMATRAALQARRGKKKSGCLVL

SEQ ID NO: 56 - protein, 127 aa, Homo sapiens
  Sm-PKN1 (SmBiT-PKN1-GBD)
MVTGYRLFEEILGGSGGGGSGGSSSGGESEPRSWSLLEQLGLAGADLAAPGVQQQLELERERLRREIRKELKLKEGAENLRRATTDLGRSLGPVELLLRGSSRRLDLLHQQLQELHAHVVLPDPAAT

SEQ ID NO: 57 - protein, 581 aa, Homo sapiens
  Lg-IP3R2-Sm (LgBiT-ITPR2-IBC-SmBiT)
MVFTLEDFVGDWEQTAAYNLDQVLEQGGVSSLLQNLAVSVTPIQRIVRSGENALKIDIHVIIPYEGLSADQMAQIEEVFKVVYPVDDHHFKVILPYGTLVIDGVTPNMLNYFGRPYEGIAVFDGKKITVTGTLWNGNKIIDERLITPDGSMLFRVTINSGGSGGGGSGGSSSGGTKYSSYREDVLKGGDVVRLFHAEQEKFLTCDEYEKKQHIFLRTTLRQSATSATSSKALWEIEVVHHDPCRGGAGQWNSLFRFKHLATGNYLAAELNPDYRDAQNEGKNVRDGVPPTSKKKRQAGEKIMYTLVSVPHGNDIASLFELDATTLQRADCLVPRNSYVRLRHLCTNTWVTSTSIPIDTDEERPVMLKIGTCQTKEDKEAFAIVSVPLSEVRDLDFANDANKVLATTVKKLENGTITQNERRFVTKLLEDLIFFVADVPNNGQEVLDVVITKPNRERQKLMREQNILAQVFGILKAPFKEKAGEGSMLRLEDLGDQRYAPYKYMLRLCYRVLRHSQQDYRKNQEYIAKNFCVMQSQIGYDILAEDTITALLHNNRKGGSGGGGSGGSSSGGVTGYRLFEEIL

SEQ ID NO: 58 - protein, 352 aa, Homo sapiens
  Gαq (∆C)
MTLESIMACCLSEEAKEARRINDEIERQLRRDKRDARRELKLLLLGTGESGKSTFIKQMRIIHGSGYSDEDKRGFTKLVYQNIFTAMQAMIRAMDTLKIPYKYEHNKAHAQLVREVDVEKVSAFENPYVDAIKSLWNDPGIQECYDRRREYQLSDSTKYYLNDLDRVADPAYLPTQQDVLRVRVPTTGIIEYPFDLQSVIFRMVDVGGQRSERRKWIHCFENVTSIMFLVALSEYDQVLVESDNENRMEESKALFRTIITYPWFQNSSVILFLNKKDLLEEKIMYSHLVDYFPEYDGPQRDAQAAREFILKMFVDLNPDSDKIIYSHFTCATDTENIRFVFAAVKDTILQLN

SEQ ID NO: 59 - protein, 359 aa, Homo sapiens
  Gαq/s
MTLESIMACCLSEEAKEARRINDEIERQLRRDKRDARRELKLLLLGTGESGKSTFIKQMRIIHGSGYSDEDKRGFTKLVYQNIFTAMQAMIRAMDTLKIPYKYEHNKAHAQLVREVDVEKVSAFENPYVDAIKSLWNDPGIQECYDRRREYQLSDSTKYYLNDLDRVADPAYLPTQQDVLRVRVPTTGIIEYPFDLQSVIFRMVDVGGQRSERRKWIHCFENVTSIMFLVALSEYDQVLVESDNENRMEESKALFRTIITYPWFQNSSVILFLNKKDLLEEKIMYSHLVDYFPEYDGPQRDAQAAREFILKMFVDLNPDSDKIIYSHFTCATDTENIRFVFAAVKDTILQLNLRQYELL

SEQ ID NO: 60 - protein, 359 aa, Homo sapiens
  Gαq/olf
MTLESIMACCLSEEAKEARRINDEIERQLRRDKRDARRELKLLLLGTGESGKSTFIKQMRIIHGSGYSDEDKRGFTKLVYQNIFTAMQAMIRAMDTLKIPYKYEHNKAHAQLVREVDVEKVSAFENPYVDAIKSLWNDPGIQECYDRRREYQLSDSTKYYLNDLDRVADPAYLPTQQDVLRVRVPTTGIIEYPFDLQSVIFRMVDVGGQRSERRKWIHCFENVTSIMFLVALSEYDQVLVESDNENRMEESKALFRTIITYPWFQNSSVILFLNKKDLLEEKIMYSHLVDYFPEYDGPQRDAQAAREFILKMFVDLNPDSDKIIYSHFTCATDTENIRFVFAAVKDTILQLNLKQYELL

SEQ ID NO: 61 - protein, 359 aa, Homo sapiens
  Gαq/i1
MTLESIMACCLSEEAKEARRINDEIERQLRRDKRDARRELKLLLLGTGESGKSTFIKQMRIIHGSGYSDEDKRGFTKLVYQNIFTAMQAMIRAMDTLKIPYKYEHNKAHAQLVREVDVEKVSAFENPYVDAIKSLWNDPGIQECYDRRREYQLSDSTKYYLNDLDRVADPAYLPTQQDVLRVRVPTTGIIEYPFDLQSVIFRMVDVGGQRSERRKWIHCFENVTSIMFLVALSEYDQVLVESDNENRMEESKALFRTIITYPWFQNSSVILFLNKKDLLEEKIMYSHLVDYFPEYDGPQRDAQAAREFILKMFVDLNPDSDKIIYSHFTCATDTENIRFVFAAVKDTILQLNLKDCGLF

SEQ ID NO: 62 - protein, 359 aa, Homo sapiens
  Gαq/i3
MTLESIMACCLSEEAKEARRINDEIERQLRRDKRDARRELKLLLLGTGESGKSTFIKQMRIIHGSGYSDEDKRGFTKLVYQNIFTAMQAMIRAMDTLKIPYKYEHNKAHAQLVREVDVEKVSAFENPYVDAIKSLWNDPGIQECYDRRREYQLSDSTKYYLNDLDRVADPAYLPTQQDVLRVRVPTTGIIEYPFDLQSVIFRMVDVGGQRSERRKWIHCFENVTSIMFLVALSEYDQVLVESDNENRMEESKALFRTIITYPWFQNSSVILFLNKKDLLEEKIMYSHLVDYFPEYDGPQRDAQAAREFILKMFVDLNPDSDKIIYSHFTCATDTENIRFVFAAVKDTILQLNLKECGLY

SEQ ID NO: 63 - protein, 359 aa, Homo sapiens
  Gαq/o
MTLESIMACCLSEEAKEARRINDEIERQLRRDKRDARRELKLLLLGTGESGKSTFIKQMRIIHGSGYSDEDKRGFTKLVYQNIFTAMQAMIRAMDTLKIPYKYEHNKAHAQLVREVDVEKVSAFENPYVDAIKSLWNDPGIQECYDRRREYQLSDSTKYYLNDLDRVADPAYLPTQQDVLRVRVPTTGIIEYPFDLQSVIFRMVDVGGQRSERRKWIHCFENVTSIMFLVALSEYDQVLVESDNENRMEESKALFRTIITYPWFQNSSVILFLNKKDLLEEKIMYSHLVDYFPEYDGPQRDAQAAREFILKMFVDLNPDSDKIIYSHFTCATDTENIRFVFAAVKDTILQLNLRGCGLY

SEQ ID NO: 64 - protein, 359 aa, Homo sapiens
  Gαq/z
MTLESIMACCLSEEAKEARRINDEIERQLRRDKRDARRELKLLLLGTGESGKSTFIKQMRIIHGSGYSDEDKRGFTKLVYQNIFTAMQAMIRAMDTLKIPYKYEHNKAHAQLVREVDVEKVSAFENPYVDAIKSLWNDPGIQECYDRRREYQLSDSTKYYLNDLDRVADPAYLPTQQDVLRVRVPTTGIIEYPFDLQSVIFRMVDVGGQRSERRKWIHCFENVTSIMFLVALSEYDQVLVESDNENRMEESKALFRTIITYPWFQNSSVILFLNKKDLLEEKIMYSHLVDYFPEYDGPQRDAQAAREFILKMFVDLNPDSDKIIYSHFTCATDTENIRFVFAAVKDTILQLNLKYIGLC

SEQ ID NO: 65 - protein, 359 aa, Homo sapiens
  Gαq
MTLESIMACCLSEEAKEARRINDEIERQLRRDKRDARRELKLLLLGTGESGKSTFIKQMRIIHGSGYSDEDKRGFTKLVYQNIFTAMQAMIRAMDTLKIPYKYEHNKAHAQLVREVDVEKVSAFENPYVDAIKSLWNDPGIQECYDRRREYQLSDSTKYYLNDLDRVADPAYLPTQQDVLRVRVPTTGIIEYPFDLQSVIFRMVDVGGQRSERRKWIHCFENVTSIMFLVALSEYDQVLVESDNENRMEESKALFRTIITYPWFQNSSVILFLNKKDLLEEKIMYSHLVDYFPEYDGPQRDAQAAREFILKMFVDLNPDSDKIIYSHFTCATDTENIRFVFAAVKDTILQLNLKEYNLV

SEQ ID NO: 66 - protein, 359 aa, Homo sapiens
  Gαq/14
MTLESIMACCLSEEAKEARRINDEIERQLRRDKRDARRELKLLLLGTGESGKSTFIKQMRIIHGSGYSDEDKRGFTKLVYQNIFTAMQAMIRAMDTLKIPYKYEHNKAHAQLVREVDVEKVSAFENPYVDAIKSLWNDPGIQECYDRRREYQLSDSTKYYLNDLDRVADPAYLPTQQDVLRVRVPTTGIIEYPFDLQSVIFRMVDVGGQRSERRKWIHCFENVTSIMFLVALSEYDQVLVESDNENRMEESKALFRTIITYPWFQNSSVILFLNKKDLLEEKIMYSHLVDYFPEYDGPQRDAQAAREFILKMFVDLNPDSDKIIYSHFTCATDTENIRFVFAAVKDTILQLNLREFNLV

SEQ ID NO: 67 - protein, 359 aa, Homo sapiens
  Gαq/16
MTLESIMACCLSEEAKEARRINDEIERQLRRDKRDARRELKLLLLGTGESGKSTFIKQMRIIHGSGYSDEDKRGFTKLVYQNIFTAMQAMIRAMDTLKIPYKYEHNKAHAQLVREVDVEKVSAFENPYVDAIKSLWNDPGIQECYDRRREYQLSDSTKYYLNDLDRVADPAYLPTQQDVLRVRVPTTGIIEYPFDLQSVIFRMVDVGGQRSERRKWIHCFENVTSIMFLVALSEYDQVLVESDNENRMEESKALFRTIITYPWFQNSSVILFLNKKDLLEEKIMYSHLVDYFPEYDGPQRDAQAAREFILKMFVDLNPDSDKIIYSHFTCATDTENIRFVFAAVKDTILQLNLDEINLL

SEQ ID NO: 68 - protein, 359 aa, Homo sapiens
  Gαq/12
MTLESIMACCLSEEAKEARRINDEIERQLRRDKRDARRELKLLLLGTGESGKSTFIKQMRIIHGSGYSDEDKRGFTKLVYQNIFTAMQAMIRAMDTLKIPYKYEHNKAHAQLVREVDVEKVSAFENPYVDAIKSLWNDPGIQECYDRRREYQLSDSTKYYLNDLDRVADPAYLPTQQDVLRVRVPTTGIIEYPFDLQSVIFRMVDVGGQRSERRKWIHCFENVTSIMFLVALSEYDQVLVESDNENRMEESKALFRTIITYPWFQNSSVILFLNKKDLLEEKIMYSHLVDYFPEYDGPQRDAQAAREFILKMFVDLNPDSDKIIYSHFTCATDTENIRFVFAAVKDTILQLNLKDIMLQ

SEQ ID NO: 69 - protein, 359 aa, Homo sapiens
  Gαq/13
MTLESIMACCLSEEAKEARRINDEIERQLRRDKRDARRELKLLLLGTGESGKSTFIKQMRIIHGSGYSDEDKRGFTKLVYQNIFTAMQAMIRAMDTLKIPYKYEHNKAHAQLVREVDVEKVSAFENPYVDAIKSLWNDPGIQECYDRRREYQLSDSTKYYLNDLDRVADPAYLPTQQDVLRVRVPTTGIIEYPFDLQSVIFRMVDVGGQRSERRKWIHCFENVTSIMFLVALSEYDQVLVESDNENRMEESKALFRTIITYPWFQNSSVILFLNKKDLLEEKIMYSHLVDYFPEYDGPQRDAQAAREFILKMFVDLNPDSDKIIYSHFTCATDTENIRFVFAAVKDTILQLNLKQLMLQ

SEQ ID NO: 70 - protein, 374 aa, Homo sapiens
  Gαs (∆C)
MGCLGNSKTEDQRNEEKAQREANKKIEKQLQKDKQVYRATHRLLLLGAGESGKSTIVKQMRILHVNGFNGDSEKATKVQDIKNNLKEAIETIVAAMSNLVPPVELANPENQFRVDYILSVMNVPDFDFPPEFYEHAKALWEDEGVRACYERSNEYQLIDCAQYFLDKIDVIKQADYVPSDQDLLRCRVLTSGIFETKFQVDKVNFHMFDVGGQRDERRKWIQCFNDVTAIIFVVASSSYNMVIREDNQTNRLQEALNLFKSIWNNRWLRTISVILFLNKQDLLAEKVLAGKSKIEDYFPEFARYTTPEDATPEPGEDPRVTRAKYFIRDEFLRISTASGDGRHYCYPHFTCAVDTENIRRVFNDCRDIIQRMHL

SEQ ID NO: 71 - protein, 380 aa, Homo sapiens
  Gαs
MGCLGNSKTEDQRNEEKAQREANKKIEKQLQKDKQVYRATHRLLLLGAGESGKSTIVKQMRILHVNGFNGDSEKATKVQDIKNNLKEAIETIVAAMSNLVPPVELANPENQFRVDYILSVMNVPDFDFPPEFYEHAKALWEDEGVRACYERSNEYQLIDCAQYFLDKIDVIKQADYVPSDQDLLRCRVLTSGIFETKFQVDKVNFHMFDVGGQRDERRKWIQCFNDVTAIIFVVASSSYNMVIREDNQTNRLQEALNLFKSIWNNRWLRTISVILFLNKQDLLAEKVLAGKSKIEDYFPEFARYTTPEDATPEPGEDPRVTRAKYFIRDEFLRISTASGDGRHYCYPHFTCAVDTENIRRVFNDCRDIIQRMHLRQYELL

SEQ ID NO: 72 - protein, 380 aa, Homo sapiens
  Gαs/i1
MGCLGNSKTEDQRNEEKAQREANKKIEKQLQKDKQVYRATHRLLLLGAGESGKSTIVKQMRILHVNGFNGDSEKATKVQDIKNNLKEAIETIVAAMSNLVPPVELANPENQFRVDYILSVMNVPDFDFPPEFYEHAKALWEDEGVRACYERSNEYQLIDCAQYFLDKIDVIKQADYVPSDQDLLRCRVLTSGIFETKFQVDKVNFHMFDVGGQRDERRKWIQCFNDVTAIIFVVASSSYNMVIREDNQTNRLQEALNLFKSIWNNRWLRTISVILFLNKQDLLAEKVLAGKSKIEDYFPEFARYTTPEDATPEPGEDPRVTRAKYFIRDEFLRISTASGDGRHYCYPHFTCAVDTENIRRVFNDCRDIIQRMHLKDCGLF

SEQ ID NO: 73 - protein, 380 aa, Homo sapiens
  Gαs/i3
MGCLGNSKTEDQRNEEKAQREANKKIEKQLQKDKQVYRATHRLLLLGAGESGKSTIVKQMRILHVNGFNGDSEKATKVQDIKNNLKEAIETIVAAMSNLVPPVELANPENQFRVDYILSVMNVPDFDFPPEFYEHAKALWEDEGVRACYERSNEYQLIDCAQYFLDKIDVIKQADYVPSDQDLLRCRVLTSGIFETKFQVDKVNFHMFDVGGQRDERRKWIQCFNDVTAIIFVVASSSYNMVIREDNQTNRLQEALNLFKSIWNNRWLRTISVILFLNKQDLLAEKVLAGKSKIEDYFPEFARYTTPEDATPEPGEDPRVTRAKYFIRDEFLRISTASGDGRHYCYPHFTCAVDTENIRRVFNDCRDIIQRMHLKECGLY

SEQ ID NO: 74 - protein, 380 aa, Homo sapiens
  Gαs/o
MGCLGNSKTEDQRNEEKAQREANKKIEKQLQKDKQVYRATHRLLLLGAGESGKSTIVKQMRILHVNGFNGDSEKATKVQDIKNNLKEAIETIVAAMSNLVPPVELANPENQFRVDYILSVMNVPDFDFPPEFYEHAKALWEDEGVRACYERSNEYQLIDCAQYFLDKIDVIKQADYVPSDQDLLRCRVLTSGIFETKFQVDKVNFHMFDVGGQRDERRKWIQCFNDVTAIIFVVASSSYNMVIREDNQTNRLQEALNLFKSIWNNRWLRTISVILFLNKQDLLAEKVLAGKSKIEDYFPEFARYTTPEDATPEPGEDPRVTRAKYFIRDEFLRISTASGDGRHYCYPHFTCAVDTENIRRVFNDCRDIIQRMHLRGCGLY

SEQ ID NO: 75 - protein, 380 aa, Homo sapiens
  Gαs/z
MGCLGNSKTEDQRNEEKAQREANKKIEKQLQKDKQVYRATHRLLLLGAGESGKSTIVKQMRILHVNGFNGDSEKATKVQDIKNNLKEAIETIVAAMSNLVPPVELANPENQFRVDYILSVMNVPDFDFPPEFYEHAKALWEDEGVRACYERSNEYQLIDCAQYFLDKIDVIKQADYVPSDQDLLRCRVLTSGIFETKFQVDKVNFHMFDVGGQRDERRKWIQCFNDVTAIIFVVASSSYNMVIREDNQTNRLQEALNLFKSIWNNRWLRTISVILFLNKQDLLAEKVLAGKSKIEDYFPEFARYTTPEDATPEPGEDPRVTRAKYFIRDEFLRISTASGDGRHYCYPHFTCAVDTENIRRVFNDCRDIIQRMHLKYIGLC

SEQ ID NO: 76 - protein, 380 aa, Homo sapiens
  Gαs/q
MGCLGNSKTEDQRNEEKAQREANKKIEKQLQKDKQVYRATHRLLLLGAGESGKSTIVKQMRILHVNGFNGDSEKATKVQDIKNNLKEAIETIVAAMSNLVPPVELANPENQFRVDYILSVMNVPDFDFPPEFYEHAKALWEDEGVRACYERSNEYQLIDCAQYFLDKIDVIKQADYVPSDQDLLRCRVLTSGIFETKFQVDKVNFHMFDVGGQRDERRKWIQCFNDVTAIIFVVASSSYNMVIREDNQTNRLQEALNLFKSIWNNRWLRTISVILFLNKQDLLAEKVLAGKSKIEDYFPEFARYTTPEDATPEPGEDPRVTRAKYFIRDEFLRISTASGDGRHYCYPHFTCAVDTENIRRVFNDCRDIIQRMHLKEYNLV

SEQ ID NO: 77 - protein, 380 aa, Homo sapiens
  Gαs/14
MGCLGNSKTEDQRNEEKAQREANKKIEKQLQKDKQVYRATHRLLLLGAGESGKSTIVKQMRILHVNGFNGDSEKATKVQDIKNNLKEAIETIVAAMSNLVPPVELANPENQFRVDYILSVMNVPDFDFPPEFYEHAKALWEDEGVRACYERSNEYQLIDCAQYFLDKIDVIKQADYVPSDQDLLRCRVLTSGIFETKFQVDKVNFHMFDVGGQRDERRKWIQCFNDVTAIIFVVASSSYNMVIREDNQTNRLQEALNLFKSIWNNRWLRTISVILFLNKQDLLAEKVLAGKSKIEDYFPEFARYTTPEDATPEPGEDPRVTRAKYFIRDEFLRISTASGDGRHYCYPHFTCAVDTENIRRVFNDCRDIIQRMHLREFNLV

SEQ ID NO: 78 - protein, 380 aa, Homo sapiens
  Gαs/16
MGCLGNSKTEDQRNEEKAQREANKKIEKQLQKDKQVYRATHRLLLLGAGESGKSTIVKQMRILHVNGFNGDSEKATKVQDIKNNLKEAIETIVAAMSNLVPPVELANPENQFRVDYILSVMNVPDFDFPPEFYEHAKALWEDEGVRACYERSNEYQLIDCAQYFLDKIDVIKQADYVPSDQDLLRCRVLTSGIFETKFQVDKVNFHMFDVGGQRDERRKWIQCFNDVTAIIFVVASSSYNMVIREDNQTNRLQEALNLFKSIWNNRWLRTISVILFLNKQDLLAEKVLAGKSKIEDYFPEFARYTTPEDATPEPGEDPRVTRAKYFIRDEFLRISTASGDGRHYCYPHFTCAVDTENIRRVFNDCRDIIQRMHLDEINLL

SEQ ID NO: 79 - protein, 380 aa, Homo sapiens
  Gαs/12
MGCLGNSKTEDQRNEEKAQREANKKIEKQLQKDKQVYRATHRLLLLGAGESGKSTIVKQMRILHVNGFNGDSEKATKVQDIKNNLKEAIETIVAAMSNLVPPVELANPENQFRVDYILSVMNVPDFDFPPEFYEHAKALWEDEGVRACYERSNEYQLIDCAQYFLDKIDVIKQADYVPSDQDLLRCRVLTSGIFETKFQVDKVNFHMFDVGGQRDERRKWIQCFNDVTAIIFVVASSSYNMVIREDNQTNRLQEALNLFKSIWNNRWLRTISVILFLNKQDLLAEKVLAGKSKIEDYFPEFARYTTPEDATPEPGEDPRVTRAKYFIRDEFLRISTASGDGRHYCYPHFTCAVDTENIRRVFNDCRDIIQRMHLKDIMLQ

SEQ ID NO: 80 - protein, 380 aa, Homo sapiens
  Gαs/13
MGCLGNSKTEDQRNEEKAQREANKKIEKQLQKDKQVYRATHRLLLLGAGESGKSTIVKQMRILHVNGFNGDSEKATKVQDIKNNLKEAIETIVAAMSNLVPPVELANPENQFRVDYILSVMNVPDFDFPPEFYEHAKALWEDEGVRACYERSNEYQLIDCAQYFLDKIDVIKQADYVPSDQDLLRCRVLTSGIFETKFQVDKVNFHMFDVGGQRDERRKWIQCFNDVTAIIFVVASSSYNMVIREDNQTNRLQEALNLFKSIWNNRWLRTISVILFLNKQDLLAEKVLAGKSKIEDYFPEFARYTTPEDATPEPGEDPRVTRAKYFIRDEFLRISTASGDGRHYCYPHFTCAVDTENIRRVFNDCRDIIQRMHLKQLMLQ

SEQ ID NO: 81 - protein, 6 aa, Homo sapiens
  C-terminally substituted 6-amino acids of Gαq/s
RQYELL

SEQ ID NO: 82 - protein, 6 aa, Homo sapiens
  C-terminally substituted 6-amino acids of Gαq/olf, Gαs/olf
KQYELL

SEQ ID NO: 83 - protein, 6 aa, Homo sapiens
  C-terminally substituted 6-amino acids of Gαq/i1, Gαs/i1
KDCGLF

SEQ ID NO: 84 - protein, 6 aa, Homo sapiens
  C-terminally substituted 6-amino acids of Gαq/i3, Gαs/i3
KECGLY

SEQ ID NO: 85 - protein, 6 aa, Homo sapiens
  C-terminally substituted 6-amino acids of Gαq/o, Gαs/o
RGCGLY

SEQ ID NO: 86 - protein, 6 aa, Homo sapiens
  C-terminally substituted 6-amino acids of Gαq/z, Gαs/z
KYIGLC

SEQ ID NO: 87 - protein, 6 aa, Homo sapiens
  C-terminally substituted 6-amino acids of Gαq/14, Gαs/14
REFNLV

SEQ ID NO: 88 - protein, 6 aa, Homo sapiens
  C-terminally substituted 6-amino acids of Gαq/16, Gαs/16
DEINLL

SEQ ID NO: 89 - protein, 6 aa, Homo sapiens
  C-terminally substituted 6-amino acids of Gαq/12
KDIMLQ

SEQ ID NO: 90 - protein, 6 aa, Homo sapiens
  C-terminally substituted 6-amino acids of Gαq/13, Gαs/13
KQLMLQ

SEQ ID NO: 91 - protein, 6 aa, Homo sapiens
  C-terminally substituted 6-amino acids of Gαs/q
KEYNLV

SEQ ID NO: 92 - protein, 6 aa, Homo sapiens
  C-terminally substituted 6-amino acids of Gαs/12
KDIMLQ

SEQ ID NO: 93 - protein, 651 aa, Homo sapiens
  amino acid sequence of the AP-TGFα.
MVPSAGQLALFALGIVLAACQALENSTSPLSADPPVAAAVVSRSGIIPVEEENPDFWNREAAEALGAAKKLQPAQTAAKNLIIFLGDGMGVSTVTAARILKGQKKDKLGPEIPLAMDRFPYVALSKTYNVDKHVPDSGATATAYLCGVKGNFQTIGLSAAARFNQCNTTRGNEVISVMNRAKKAGKSVGVVTTTRVQHASPAGTYAHTVNRNWYSDADVPASARQEGCQDIATQLISNMDIDVILGGGRKYMFRMGTPDPEYPDDYSQGGTRLDGKNLVQEWLAKRQGARYVWNRTELMQASLDPSVTHLMGLFEPGDMKYEIHRDSTLDPSLMEMTEAALRLLSRNPRGFFLFVEGGRIDHGHHESRAYRALTETIMFDDAIERAGQLTSEEDTLSLVTADHSHVFSFGGYPLRGSSIFGLAPGKARDRKAYTVLLYGNGPGYVLKDGARPDVTESESGSPEYRQQSAVPLDEETHAGEDVAVFARGPQAHLVHGVQEQTFIAHVMAFAACLEPYTACDLAPPAGTTDAAHPGYHDCPDSHTQFCFHGTCRFLVQEDKPACVCHSGYVGARCEHADLLAVVAASQKKQAITALVVVSIVALAVLIITCVLIHCCQVRKHCEWCRALICRHEKPSALLKGRTACCHSETVV

SEQ ID NO: 94 - protein, 39 aa, Homo sapiens
  signal-sequence peptide and the cleaved fragment of human TGFA
MVPSAGQLALFALGIVLAACQALENSTSPLSADPPVAAA

SEQ ID NO: 95 - protein, 489 aa, Homo sapiens
  alkaline phosphatase sequence derived from human ALPP
GIIPVEEENPDFWNREAAEALGAAKKLQPAQTAAKNLIIFLGDGMGVSTVTAARILKGQKKDKLGPEIPLAMDRFPYVALSKTYNVDKHVPDSGATATAYLCGVKGNFQTIGLSAAARFNQCNTTRGNEVISVMNRAKKAGKSVGVVTTTRVQHASPAGTYAHTVNRNWYSDADVPASARQEGCQDIATQLISNMDIDVILGGGRKYMFRMGTPDPEYPDDYSQGGTRLDGKNLVQEWLAKRQGARYVWNRTELMQASLDPSVTHLMGLFEPGDMKYEIHRDSTLDPSLMEMTEAALRLLSRNPRGFFLFVEGGRIDHGHHESRAYRALTETIMFDDAIERAGQLTSEEDTLSLVTADHSHVFSFGGYPLRGSSIFGLAPGKARDRKAYTVLLYGNGPGYVLKDGARPDVTESESGSPEYRQQSAVPLDEETHAGEDVAVFARGPQAHLVHGVQEQTFIAHVMAFAACLEPYTACDLAPPAGTTDAAHP

SEQ ID NO: 96 - protein, 48 aa, Homo sapiens
  mature, ectodomain-shed fragment of human TGFA
GYHDCPDSHTQFCFHGTCRFLVQEDKPACVCHSGYVGARCEHADLLAV